European Patent Specification EP 3 988 565 B1, published July 22, 2026. Title: T CELL RECEPTORS. Applicant: ADAPTIMMUNE LIMITED. Application PCT/EP2017/058580. The sequence listing filed with the application follows.

SEQUENCE LISTING (29 sequences)

SEQ ID NO: 1 - protein, 10 aa, Homo sapiens
GVYDGREHTV

SEQ ID NO: 2 - protein, 10 aa, Homo sapiens
GVYDGEEHSV

SEQ ID NO: 3 - protein, 105 aa, Artificial Sequence
  source: /note="Description of Artificial Sequence: Synthetic polypeptide"
MKNQVEQSPQSLIILEGKNCTLQCNYTVSPFSNLRWYKQDTGRGPVSLTIMTFSENTKSNGRYTATLDADTKQSSLHITASQLSDSASYICVVSGGTDSWGKLQF

SEQ ID NO: 4 - protein, 123 aa, Artificial Sequence
  source: /note="Description of Artificial Sequence: Synthetic polypeptide"
MASLLFFCGAFYLLGTGSMDADVTQTPRNRITKTGKRIMLECSQTKGHDRMYWYRQDPGLGLRLIYYSFDVKDINKGEISDGYSVSRQAQAKFSLSLESAIPNQTALYFCATSGQGAYNEQFF

SEQ ID NO: 5 - protein, 229 aa, Artificial Sequence
  source: /note="Description of Artificial Sequence: Synthetic polypeptide"
MKKHLTTFLVILWLYFYRGNGKNQVEQSPQSLIILEGKNCTLQCNYTVSPFSNLRWYKQDTGRGPVSLTIMTFSENTKSNGRYTATLDADTKQSSLHITASQLSDSASYICVVSGGTDSWGKLQFGAGTQVVVTPDIQNPDPAVYQLRDSKSSDKSVCLFTDFDSQTNVSQSKDSDVYITDKTVLDMRSMDFKSNSAVAWSNKSDFACANAFNNSIIPEDTFFPSPESS

SEQ ID NO: 6 - protein, 262 aa, Artificial Sequence
  source: /note="Description of Artificial Sequence: Synthetic polypeptide"
MASLLFFCGAFYLLGTGSMDADVTQTPRNRITKTGKRIMLECSQTKGHDRMYWYRQDPGLGLRLIYYSFDVKDINKGEISDGYSVSRQAQAKFSLSLESAIPNQTALYFCATSGQGAYNEQFFGPGTRLTVLEDLKNVFPPEVAVFEPSEAEISHTQKATLVCLATGFYPDHVELSWWVNGKEVHSGVSTDPQPLKEQPALNDSRYCLSSRLRVSATFWQNPRNHFRCQVQFYGLSENDEWTQDRAKPVTQIVSAEAWGRAD

SEQ ID NO: 7 - protein, 105 aa, Artificial Sequence
  source: /note="Description of Artificial Sequence: Synthetic polypeptide"
MKNQVEQSPQSLIILEGKNCTLQCNYTVSPFSNLRWYKQDTGRGPVSLTIVTFSENTKSNGRYTATLDADTKQSSLHITASQLSDSASYICVVSGGTDSWGKLQF

SEQ ID NO: 8 - protein, 105 aa, Artificial Sequence
  source: /note="Description of Artificial Sequence: Synthetic polypeptide"
MKNQVEQSPQSLIILEGKNCTLQCNYTVSPFSNLRWYKQDTGRGPVSLTILTFSENTKSNGRYTATLDADTKQSSLHITASQLSDSASYICVVSGGTDSWGKLQF

SEQ ID NO: 9 - protein, 123 aa, Artificial Sequence
  source: /note="Description of Artificial Sequence: Synthetic polypeptide"
MASLLFFCGAFYLLGTGSMDADVTQTPRNRITKTGKRIMLECSQTKGHDRMYWYRQDPGLGLRLIYYSFDVKDINKGEISDGYSVSRQAQAKFSLSLESAIPNQTALYFCATSGQGAYEEQFF

SEQ ID NO: 10 - protein, 271 aa, Artificial Sequence
  source: /note="Description of Artificial Sequence: Synthetic polypeptide"
METLLGLLILWLQLQWVSSKQEVTQIPAALSVPEGENLVLNCSFTDSAIYNLQWFRQDPGKGLTSLLLIQSSQREQTSGRLNASLDKSSGRSTLYIAASQPGDSATYLCAVGGYSTLTFGKGTVLLVSPDNIQNPDPAVYQLRDSKSSDKSVCLFTDFDSQTNVSQSKDSDVYITDKTVLDMRSMDFKSNSAVAWSNKSDFACANAFNNSIIPEDTFFPSPESSCDVKLVEKSFETDTNLNFQNLSVIGFRILLLKVAGFNLLMTLRLWSS

SEQ ID NO: 11 - protein, 308 aa, Artificial Sequence
  source: /note="Description of Artificial Sequence: Synthetic polypeptide"
MSISLLCCAAFPLLWAGPVNAGVTQTPKFRILKIGQSMTLQCAQDMNHNYMYWYRQDPGMGLKLIYYSVGAGITDKGEVPNGYNVSRSTTEDFPLRLELAAPSQTSVYFCASSYSRWSPLHFGNGTRLTVTEDLNKVFPPEVAVFEPSEAEISHTQKATLVCLATGFFPDHVELSWWVNGKEVHSGVSTDPQPLKEQPALNDSRYCLSSRLRVSATFWQNPRNHFRCQVQFYGLSENDEWTQDRAKPVTQIVSAEAWGRADCGFTSVSYQQGVLSATILYEILLGKATLYAVLVSALVLMAMVKRKDF

SEQ ID NO: 12 - protein, 208 aa, Artificial Sequence
  source: /note="Description of Artificial Sequence: Synthetic polypeptide"
MQKEVEQNSGPLSVPEGAIASLNCTYSDRGSQSFFWYRQYSGKSPELIMFIYSNGDKEDGRFTAQLNKASQYVSLLIRDSQPSDSATYLCAVKMANQAGTALIFGKGTTLSVSSNIQNPDPAVYQLRDSKSSDKSVCLFTDFDSQTNVSQSKDSDVYITDKCVLDMRSMDFKSNSAVAWSNKSDFACANAFNNSIIPEDTFFPSPESS

SEQ ID NO: 13 - protein, 244 aa, Artificial Sequence
  source: /note="Description of Artificial Sequence: Synthetic polypeptide"
MQDGGITQSPKFQVLRTGQSMTLLCAQDMNHEYMYWYRQDPGMGLRLIHYSVGAGITDQGEVPNGYNVSRLNKREFSLRLESAAPSQTSVYFCASLGGLADEQFFGPGTRLTVLEDLKNVFPPEVAVFEPSEAEISHTQKATLVCLATGFYPDHVELSWWVNGKEVHSGVCTDPQPLKEQPALNDSRYALSSRLRVSATFWQDPRNHFRCQVQFYGLSENDEWTQDRAKPVTQIVSAEAWGRAD

SEQ ID NO: 14 - protein, 275 aa, Artificial Sequence
  source: /note="Description of Artificial Sequence: Synthetic polypeptide"
MKTFAGFSFLFLWLQLDCMSRGEDVEQSLFLSVREGDSSVINCTYTDSSSTYLYWYKQEPGAGLQLLTYIFSNMDMKQDQRLTVLLNKKDKHLSLRIADTQTGDSAIYFCAERNSGAGSYQLTFGKGTKLSVIPNIQNPDPAVYQLRDSKSSDKSVCLFTDFDSQTNVSQSKDSDVYITDKTVLDMRSMDFKSNSAVAWSNKSDFACANAFNNSIIPEDTFFPSPESSCDVKLVEKSFETDTNLNFQNLSVIGFRILLLKVAGFNLLMTLRLWSS

SEQ ID NO: 15 - protein, 311 aa, Artificial Sequence
  source: /note="Description of Artificial Sequence: Synthetic polypeptide"
MGTSLLCWMALCLLGADHADTGVSQNPRHKITKRGQNVTFRCDPISEHNRLYWYRQTLGQGPEFLTYFQNEAQLEKSRLLSDRFSAERPKGSFSTLEIQRTEQGDSAMYLCASSLFSGVNTEAFFGQGTRLTVVEDLNKVFPPEVAVFEPSEAEISHTQKATLVCLATGFFPDHVELSWWVNGKEVHSGVSTDPQPLKEQPALNDSRYCLSSRLRVSATFWQNPRNHFRCQVQFYGLSENDEWTQDRAKPVTQIVSAEAWGRADCGFTSVSYQQGVLSATILYEILLGKATLYAVLVSALVLMAMVKRKDF

SEQ ID NO: 16 - protein, 10 aa, Homo sapiens
GVVDGREHTV

SEQ ID NO: 17 - protein, 10 aa, Homo sapiens
GVYDGAYVSV

SEQ ID NO: 18 - protein, 6 aa, Artificial Sequence
  source: /note="Description of Artificial Sequence: Synthetic peptide"
VSPFSN

SEQ ID NO: 19 - protein, 6 aa, Artificial Sequence
  source: /note="Description of Artificial Sequence: Synthetic peptide"
LTIMTF

SEQ ID NO: 20 - protein, 6 aa, Artificial Sequence
  source: /note="Description of Artificial Sequence: Synthetic peptide"
LTRMTF

SEQ ID NO: 21 - protein, 6 aa, Artificial Sequence
  source: /note="Description of Artificial Sequence: Synthetic peptide"
LTIVTF

SEQ ID NO: 22 - protein, 6 aa, Artificial Sequence
  source: /note="Description of Artificial Sequence: Synthetic peptide"
LTILTF

SEQ ID NO: 23 - protein, 15 aa, Artificial Sequence
  source: /note="Description of Artificial Sequence: Synthetic peptide"
CVVSGGTDSWGKLQF

SEQ ID NO: 24 - protein, 5 aa, Artificial Sequence
  source: /note="Description of Artificial Sequence: Synthetic peptide"
KGHDR

SEQ ID NO: 25 - protein, 5 aa, Artificial Sequence
  source: /note="Description of Artificial Sequence: Synthetic peptide"
SVFDK

SEQ ID NO: 26 - protein, 14 aa, Artificial Sequence
  source: /note="Description of Artificial Sequence: Synthetic peptide"
CATSGQGAYNEQFF

SEQ ID NO: 27 - protein, 14 aa, Artificial Sequence
  source: /note="Description of Artificial Sequence: Synthetic peptide"
CATSGQGAYREQFF

SEQ ID NO: 28 - protein, 9 aa, Homo sapiens
GVDGKSDSV

SEQ ID NO: 29 - protein, 5 aa, Artificial Sequence
  source: /note="Description of Artificial Sequence: Synthetic peptide"
SFDVK